European Patent Application EP 4 663 765 A1, published December 17, 2025. Title: Methods of manufacturing compositions containing processed unsaturated fatty acids and their applications. Applicant: AMANO ENZYME INC. The sequence listing filed with the application follows.

SEQUENCE LISTING (2 sequences)

SEQ ID NO: 1 - protein, 413 aa, Exiguobacterium sp. AT1b
MGKVIPKQEGLDHSVDFLREGYLFVANRRKSFQSNIFESRLLGERVICLGGEEAAEVFYDANKFTRQDAAPKRLLKTLFGEGGVQTLDGSEHTHRKQMFMSLMTKENIDRLLRLTYREWNQIERMGEEIVLYDIAQEVLMKAVCEWSGVPLAKEEVGKRTEEMRLLFESGTSLGPTYLQGRKARSSAEVWIRQMVKEVRSNRLLPNEHTALYEFSWHRDESGELLPEEVVAVEVLNILRPTVAISVYVLFTVLALHQFPDVKEQVERGEVSKTEFVQEVRRFYPFFPVAAARVKTDFEWDGYAFPEGTLTLLDLYGTNHDVSIWTEPDRFDPSRFKDWKESPFNFIPQGGGDVDFGHRCAGEHVTIAILAQVIELFTKEYAYTVPPQDLSYSFVDMPSLPKSKLRLTHLTRNQ

SEQ ID NO: 2 - DNA, 1242 bp, synthetic construct
  source 1..1242: mol_type = other DNA
atgggtaaagttatcccgaaacaggaaggcctggatcactctgtggactttctgcgcgagggctatctgtttgtggcaaaccgccgtaaatctttccagtctaacatcttcgagagccgcctgctgggcgagcgtgttatctgcctgggtggcgaagaagctgcagaggtgttttatgacgcgaacaaattcacccgtcaggacgcggcaccgaaacgtctgctgaaaaccctgttcggtgaaggcggtgtgcagaccctggacggttccgaacacacccaccgcaagcagatgttcatgagcctgatgaccaaagaaaacattgatcgcctgctgcgcctgacttatcgtgaatggaaccagatcgaacgtatgggtgaggaaatcgttctgtacgacatcgcacaggaggtgctgatgaaagcagtgtgcgaatggtctggtgttccgctggctaaggaagaagtgggtaagcgtaccgaagaaatgcgtctgctgttcgaatctggtacctctctgggtccgacctatctgcagggtcgcaaagcgcgttcttctgcggaagtttggattcgtcagatggttaaagaagttcgctctaaccgtctgctgccgaacgaacatactgcgctgtatgaattctcttggcaccgtgatgagagcggtgaactgctgccggaagaggtggtggctgttgaagtgctgaacattctgcgtccgactgttgctatctctgtgtacgtgctgtttaccgtgctggcgctgcaccagtttccggacgttaaggaacaggttgagcgtggtgaggtttctaaaactgagtttgtgcaggaagtgcgccgtttctacccgtttttcccggttgcagcagctcgtgttaaaaccgatttcgaatgggatggctatgcgttcccggaaggtaccctgactctgctggacctgtacggtactaaccacgacgtgtctatttggaccgaaccggatcgtttcgacccgtctcgtttcaaagattggaaagaatctccgttcaacttcatcccgcagggcggtggtgatgttgattttggccaccgttgcgcgggtgagcacgttaccatcgcaatcctggcgcaggttatcgaactgttcaccaaggagtatgcgtataccgttccgccgcaggatctgtcttactctttcgttgacatgccgtccctgccgaaaagcaaactgcgtctgactcacctgacccgtaaccagtaa